European Patent Specification EP 3 708 676 B1, published October 30, 2024. Title: PRESERVATION OF FETAL NUCLEIC ACIDS IN MATERNAL PLASMA. Applicant: Streck, Inc. The sequence listing filed with the application follows.

SEQUENCE LISTING (1 sequence)

SEQ ID NO: 1 - DNA, 37 bp, Probe for SRY sequence quantification
atggctctagagaatcccagaatgcgaaactcagaga